European Patent Application EP 4 357 449 A1, published April 24, 2024. Title: Method for Producing Cerebral Cortex Cell Preparation Derived from Human Pluripotent Stem Cell. Applicant: Kyoto University Sumitomo Pharma Co., Ltd. SUMITOMO CHEMICAL COMPANY, LIMITED. The sequence listing filed with the application follows.

SEQUENCE LISTING (22 sequences)

SEQ ID NO: 1 - DNA, 20 bp, Artificial Sequence
  Forward primer for POU5F1
agaccatctgccgctttgag

SEQ ID NO: 2 - DNA, 16 bp, Artificial Sequence
  Reverse primer for POU5F1
gcaagggccgcagctt

SEQ ID NO: 3 - DNA, 25 bp, Artificial Sequence
  Forward primer for NANOG
ggctctgttttgctatatcccctaa

SEQ ID NO: 4 - DNA, 24 bp, Artificial Sequence
  Reverse primer for NANOG
cattacgatgcagcaaatacgaga

SEQ ID NO: 5 - DNA, 22 bp, Artificial Sequence
  Forward primer for BMP4
atgattcctggtaaccgaatgc

SEQ ID NO: 6 - DNA, 21 bp, Artificial Sequence
  Reverse primer for BMP4
ccccgtctcaggtatcaaact

SEQ ID NO: 7 - DNA, 20 bp, Artificial Sequence
  Forward primer for NODAL
tgagccaacaagaggatctg

SEQ ID NO: 8 - DNA, 20 bp, Artificial Sequence
  Reverse primer for NODAL
tggaaaatctcaatggcaag

SEQ ID NO: 9 - DNA, 22 bp, Artificial Sequence
  Forward primer for TGFB1
tacctgaacccgtgttgctctc

SEQ ID NO: 10 - DNA, 22 bp, Artificial Sequence
  Reverse primer for TGFB1
gttgctgaggtatcgccaggaa

SEQ ID NO: 11 - DNA, 17 bp, Artificial Sequence
  Forward primer for SOX1
gcggagctcgtcgcatt

SEQ ID NO: 12 - DNA, 27 bp, Artificial Sequence
  Reverse primer for SOX1
gcggtaacaactacaaaaaacttgtaa

SEQ ID NO: 13 - DNA, 21 bp, Artificial Sequence
  Forward primer for PAX6
ctggctagcgaaaagcaacag

SEQ ID NO: 14 - DNA, 25 bp, Artificial Sequence
  Reverse primer for PAX6
cccgttcaacatccttagtttatca

SEQ ID NO: 15 - DNA, 19 bp, Artificial Sequence
  Forward primer for T (TBXT)
atggaggaacccggagaca

SEQ ID NO: 16 - DNA, 20 bp, Artificial Sequence
  Reverse primer for T (TBXT)
tgaggatttgcaggtggaca

SEQ ID NO: 17 - DNA, 26 bp, Artificial Sequence
  Forward primer for SOX17
cgctttcatggtgtgggctaaggacg

SEQ ID NO: 18 - DNA, 26 bp, Artificial Sequence
  Reverse primer for SOX17
tagttggggtggtcctgcatgtgctg

SEQ ID NO: 19 - DNA, 21 bp, Artificial Sequence
  Forward primer for hCGalpha
accgccctgaacacatcctgc

SEQ ID NO: 20 - DNA, 23 bp, Artificial Sequence
  Reverse primer for hCGalpha
gcgtgcattctgggcaatcctgc

SEQ ID NO: 21 - DNA, 21 bp, Artificial Sequence
  Forward primer for SOX2
gccgagtggaaacttttgtcg

SEQ ID NO: 22 - DNA, 22 bp, Artificial Sequence
  Reverse primer for SOX2
ggcagcgtgtacttatccttct